European Patent Specification EP 3 558 265 B1, published April 16, 2025. Title: INTERPENTRATING MICROSTRUCTURES FOR NANOCHANNEL-BASED CARGO DELIVERY. Applicant: Ohio State Innovation Foundation. The sequence listing filed with the application follows.

SEQUENCE LISTING (29 sequences)

SEQ ID NO: 1 - DNA, 21 bp, Artificial Sequence
  Synthetic Construct
ctctgctgcctcctggcttct

SEQ ID NO: 2 - DNA, 21 bp, Artificial Sequence
  Synthetic Construct
cgaggcggatcacaagcaata

SEQ ID NO: 3 - DNA, 19 bp, Artificial Sequence
  Synthetic Construct
tcaatgggcgggggtcgtt

SEQ ID NO: 4 - DNA, 23 bp, Artificial Sequence
  Synthetic Construct
gcggtctggcagtaaaaactatc

SEQ ID NO: 5 - DNA, 23 bp, Artificial Sequence
  Synthetic Construct
gtgaaacagcattgctgtcactt

SEQ ID NO: 6 - DNA, 19 bp, Artificial Sequence
  Synthetic Construct
cgacgagggatcctacgac

SEQ ID NO: 7 - DNA, 18 bp, Artificial Sequence
  Synthetic Construct
cttcctctgccctcgaac

SEQ ID NO: 8 - DNA, 22 bp, Artificial Sequence
  Synthetic Construct
ggtggagttcaagtccatctac

SEQ ID NO: 9 - DNA, 20 bp, Artificial Sequence
  Synthetic Construct
tggcgtccacgtagtagtag

SEQ ID NO: 10 - DNA, 22 bp, Artificial Sequence
  Synthetic Construct
atacaagagctgttcagctgtc

SEQ ID NO: 11 - DNA, 20 bp, Artificial Sequence
  Synthetic Construct
gtcgtgcatatttgccactg

SEQ ID NO: 12 - DNA, 20 bp, Artificial Sequence
  Synthetic Construct
ggaccagtccccgaagcagc

SEQ ID NO: 13 - DNA, 20 bp, Artificial Sequence
  Synthetic Construct
agtggagcagctggcctgga

SEQ ID NO: 14 - DNA, 20 bp, Artificial Sequence
  Synthetic Construct
agcgctgtgaacgcttgcct

SEQ ID NO: 15 - DNA, 20 bp, Artificial Sequence
  Synthetic Construct
catgagaggccctcccggct

SEQ ID NO: 16 - DNA, 17 bp, Artificial Sequence
  Synthetic Construct
ccgtccagctcgaccag

SEQ ID NO: 17 - DNA, 18 bp, Artificial Sequence
  Synthetic Construct
gatcacatggtcctgctg

SEQ ID NO: 18 - DNA, 20 bp, Artificial Sequence
  Synthetic Construct
gtgcaacgagcagggcgagt

SEQ ID NO: 19 - DNA, 20 bp, Artificial Sequence
  Synthetic Construct
ggagccaccgcgcacagaat

SEQ ID NO: 20 - DNA, 20 bp, Artificial Sequence
  Synthetic Construct
gctggtgcagagcggcaaga

SEQ ID NO: 21 - DNA, 20 bp, Artificial Sequence
  Synthetic Construct
agacggcggtaggtggcgat

SEQ ID NO: 22 - DNA, 20 bp, Artificial Sequence
  Synthetic Construct
tacacgggcgagggcatgga

SEQ ID NO: 23 - DNA, 20 bp, Artificial Sequence
  Synthetic Construct
tcacttgggcccctgggctt

SEQ ID NO: 24 - DNA, 24 bp, Artificial Sequence
  Synthetic Construct
gtgtgatgggattccctggaccta

SEQ ID NO: 25 - DNA, 24 bp, Artificial Sequence
  Synthetic Construct
cctgagctccagcttctccatctt

SEQ ID NO: 26 - DNA, 20 bp, Artificial Sequence
  Synthetic Construct
aggccaggtggtggacgtgt

SEQ ID NO: 27 - DNA, 20 bp, Artificial Sequence
  Synthetic Construct
cacgctggacctgcttgggg

SEQ ID NO: 28 - DNA, 20 bp, Artificial Sequence
  Synthetic Construct
gtgcagtgccagcctcgtcc

SEQ ID NO: 29 - DNA, 20 bp, Artificial Sequence
  Synthetic Construct
gcaccggcctcaccccattt